European Patent Application EP 4 434 544 A1, published September 25, 2024. Title: CD300LD INHIBITOR AND USE THEREOF IN THE PREPARATION OF TUMOR IMMUNOTHERAPY PRODUCTS. Applicant: FUDAN UNIVERSITY. Application WO. The sequence listing filed with the application follows.

SEQUENCE LISTING (34 sequences)

SEQ ID NO: 1 - DNA, 21 bp, synthetic construct
  source 1..21: mol_type = other DNA
acattgaccaagccccaaaaa

SEQ ID NO: 2 - DNA, 21 bp, synthetic construct
  source 1..21: mol_type = other DNA
agcaggggtaactccacaaag

SEQ ID NO: 3 - DNA, 24 bp, synthetic construct
  source 1..24: mol_type = other DNA
gtctacatgttccagtatgactcc

SEQ ID NO: 4 - DNA, 25 bp, synthetic construct
  source 1..25: mol_type = other DNA
agtgagttgtcatatttctcgtggt

SEQ ID NO: 5 - DNA, 20 bp, synthetic construct
  source 1..20: mol_type = other DNA
tcccaggttactccattgcc

SEQ ID NO: 6 - DNA, 20 bp, synthetic construct
  source 1..20: mol_type = other DNA
gcctgagccataagcacact

SEQ ID NO: 7 - DNA, 21 bp, synthetic construct
  source 1..21: mol_type = other DNA
tgtgggcatcaatggatttgg

SEQ ID NO: 8 - DNA, 22 bp, synthetic construct
  source 1..22: mol_type = other DNA
acaccatgtattccgggtcaat

SEQ ID NO: 9 - DNA, 20 bp, synthetic construct
  source 1..20: mol_type = other DNA
actgctggaatgaccaatag

SEQ ID NO: 10 - DNA, 20 bp, synthetic construct
  source 1..20: mol_type = other DNA
gtttctgcatatggtacacc

SEQ ID NO: 11 - DNA, 342 bp, synthetic construct
  source 1..342: mol_type = other DNA
gctgctgcacggctcaggattcagtcacaggtccagaggaggtgagcggtcaggagcagggctccttgacagtgcagtgcagatattcctcatactggaagggttacaagaagtactggtgccgaggagttcctcagagatcatgtgatattcttgttgaaaccgataaatcagagcagctggtgaagaagaaccgtgtgtccatcagggacaaccagagagacttcatcttcacagtgaccatggaggatctgaggatgagcgatgctggcatttactggtgtggaattacgaaaggtggacctgatcccatgtttaaagttaatgtgaacattgaccaag

SEQ ID NO: 12 - DNA, 20 bp, synthetic construct
  source 1..20: mol_type = other DNA
ctcagattccacggatctga

SEQ ID NO: 13 - DNA, 20 bp, synthetic construct
  source 1..20: mol_type = other DNA
ctgtggcattcgtgtcactt

SEQ ID NO: 14 - DNA, 35 bp, synthetic construct
  source 1..35: mol_type = other DNA
tgcggccgcgaattcatgtggcagttctctgctct

SEQ ID NO: 15 - DNA, 34 bp, synthetic construct
  source 1..34: mol_type = other DNA
cctgctgagcagcatctacgtcgacatcgagggc

SEQ ID NO: 16 - DNA, 531 bp, synthetic construct
  source 1..531: mol_type = other DNA
atgtggcagttctctgctctactcctattcttcctcccaggctgctgcacggctcaggattcagtcacaggtccagaggaggtgagcggtcaggagcagggctccttgacagtgcagtgcagatattcctcatactggaagggttacaagaagtactggtgccgaggagttcctcagagatcatgtgatattcttgttgaaaccgataaatcagagcagctggtgaagaagaaccgtgtgtccatcagggacaaccagagagacttcatcttcacagtgaccatggaggatctgaggatgagcgatgctggcatttactggtgtggaattacgaaaggtggacctgatcccatgtttaaagttaatgtgaacattgaccaagccccaaaaagttcaatgatgaccaccacagccacagttctgaaatccatacaaccaagcgctgagaacactggcaaggaacaagtgactcagagcaaagaagtgactcagagcaggccccacaccaggtccctgctgagcagcatctac

SEQ ID NO: 17 - protein, 177 aa, synthetic construct
MWQFSALLLFFLPGCCTAQDSVTGPEEVSGQEQGSLTVQCRYSSYWKGYKKYWCRGVPQRSCDILVETDKSEQLVKKNRVSIRDNQRDFIFTVTMEDLRMSDAGIYWCGITKGGPDPMFKVNVNIDQAPKSSMMTTTATVLKSIQPSAENTGKEQVTQSKEVTQSRPHTRSLLSSIY

SEQ ID NO: 18 - DNA, 5387 bp, synthetic construct
  source 1..5387: mol_type = other DNA
ccattcgccattcaggctgcgcaactgttgggaagggcgatcggtgcgggcctcttcgctattacgccagctggcgaaagggggatgtgctgcaaggcgattaagttgggtaacgccagggttttcccagtcacgacgttgtaaaacgacggccagtgccaagctgatctatacattgaatcaatattggcaattagccatattagtcattggttatatagcataaatcaatattggctattggccattgcatacgttgtatctatatcataatatgtacatttatattggctcatgtccaatatgaccgccatgttgacattgattattgactagttattaatagtaatcaattacggggtcattagttcatagcccatatatggagttccgcgttacataacttacggtaaatggcccgcctggctgaccgcccaacgacccccgcccattgacgtcaataatgacgtatgttcccatagtaacgccaatagggactttccattgacgtcaatgggtggagtatttacggtaaactgcccacttggcagtacatcaagtgtatcatatgccaagtccgccccctattgacgtcaatgacggtaaatggcccgcctggcattatgcccagtacatgaccttacgggactttcctacttggcagtacatctacgtattagtcatcgctattaccatggtgatgcggttttggcagtacaccaatgggcgtggatagcggtttgactcacggggatttccaagtctccaccccattgacgtcaatgggagtttgttttggcaccaaaatcaacgggactttccaaaatgtcgtaataaccccgccccgttgacgcaaatgggcggtaggcgtgtacggtgggaggtctatataagcagagctcgtttagtgaaccgtcagaattaagcttgcggccgcgaattcatcgatagatctgatatcggtaccagtcgacatcgagggccgcatggaccccaaatcttgtaaaactcacacatgcccaccgtgcccagcacctgaactcctggggggaccgtcagtcttcctcttccccccaaaacccaaggacaccctcatgatctcccggacccctgaggtcacatgcgtggtggtggacgtgagccacgaagaccctgaggtcaagttcaactggtacgtggacggcgtggaggtgcataatgccaagacaaagccgcgggaggagcagtacaacagcacgtaccgtgtggtcagcgtcctcaccgtcctgcaccaggactggctgaatggcaaggagtacaagtgcaaggtctccaacaaagccctcccagcccccatcgagaaaaccatctccaaagccaaagggcagccccgagaaccacaggtgtacaccctgcccccatcccgggaggagatgaccaagaaccaggtcagcctgacctgcctggtcaaaggcttctatcccagcgacatcgccgtggagtgggagagcaatgggcagccggagaacaactacaagaccacgcctcccgtgctggactccgacggctccttcttcctctacagcaagctcaccgtggacaagagcaggtggcagcaggggaacgtcttctcatgctccgtgatgcacgaggctctgcacaaccactacacgcagaagagcctctccctgtctccgggtaaatgaggatcccgggctgattacaaggacgacgatgacaagtaggttgggtggcatccctgtgacccctccccagtgcctctcctggccctggaagttgccactccagtgcccaccagccttgtcctaataaaattaagttgcatcattttgtctgactaggtgtccttctataatattatggggtggaggggggtggtatggagcaaggggcaagttgggaagacaacctgtagggcctgcggggtctattgggaaccaagctggagtgcagtggcacaatcttggctcactgcaatctccgcctcctgggttcaagcgattctcctgcctcagcctcccgagttgttgggattccaggcatgcatgaccaggctcagctaatttttgtttttttggtagagacggggtttcaccatattggccaggctggtctccaactcctaatctcaggtgatctacccaccttggcctcccaaattgctgggattacaggcgtgaaccactgctcccttccctgtccttctgattttaaaataactataccagcaggaggacgtccagacacagcataggctacctggccatgcccaaccggtgggacatttgagttgcttgcttggcactgtcctctcatgcgttgggtccactcagtagatgcctgttgaattgggtacgcggccagcttggctgtggaatgtgtgtcagttagggtgtggaaagtccccaggctccccagcaggcagaagtatgcaaagcatgcatctcaattagtcagcaaccaggtgtggaaagtccccaggctccccagcaggcagaagtatgcaaagcatgcatctcaattagtcagcaaccatagtcccgcccctaactccgcccatcccgcccctaactccgcccagttccgcccattctccgccccatggctgactaattttttttatttatgcagaggccgaggccgcctcggcctctgagctattccagaagtagtgaggaggcttttttggaggcctaggcttttgcaaaaagctcctcgaggaactgaaaaaccagaaagttaattccctatagtgagtcgtattaaattcgtaatcatgtcatagctgtttcctgtgtgaaattgttatccgctcacaattccacacaacatacgagccggaagcataaagtgtaaagcctggggtgcctaatgagtgagctaactcacattaattgcgttgcgctcactgcccgctttccagtcgggaaacctgtcgtgccagctgcattaatgaatcggccaacgcgcggggagaggcggtttgcgtattgggcgctcttccgcttcctcgctcactgactcgctgcgctcggtcgttcggctgcggcgagcggtatcagctcactcaaaggcggtaatacggttatccacagaatcaggggataacgcaggaaagaacatgtgagcaaaaggccagcaaaaggccaggaaccgtaaaaaggccgcgttgctggcgtttttccataggctccgcccccctgacgagcatcacaaaaatcgacgctcaagtcagaggtggcgaaacccgacaggactataaagataccaggcgtttccccctggaagctccctcgtgcgctctcctgttccgaccctgccgcttaccggatacctgtccgcctttctcccttcgggaagcgtggcgctttctcatagctcacgctgtaggtatctcagttcggtgtaggtcgttcgctccaagctgggctgtgtgcacgaaccccccgttcagcccgaccgctgcgccttatccggtaactatcgtcttgagtccaacccggtaagacacgacttatcgccactggcagcagccactggtaacaggattagcagagcgaggtatgtaggcggtgctacagagttcttgaagtggtggcctaactacggctacactagaagaacagtatttggtatctgcgctctgctgaagccagttaccttcggaaaaagagttggtagctcttgatccggcaaacaaaccaccgctggtagcggtggtttttttgtttgcaagcagcagattacgcgcagaaaaaaaggatctcaagaagatcctttgatcttttctacggggtctgacgctcagtggaacgaaaactcacgttaagggattttggtcatgagattatcaaaaaggatcttcacctagatccttttaaattaaaaatgaagttttaaatcaatctaaagtatatatgagtaaacttggtctgacagttaccaatgcttaatcagtgaggcacctatctcagcgatctgtctatttcgttcatccatagttgcctgactccccgtcgtgtagataactacgatacgggagggcttaccatctggccccagtgctgcaatgataccgcgagacccacgctcaccggctccagatttatcagcaataaaccagccagccggaagggccgagcgcagaagtggtcctgcaactttatccgcctccatccagtctattaattgttgccgggaagctagagtaagtagttcgccagttaatagtttgcgcaacgttgttgccattgctacaggcatcgtggtgtcacgctcgtcgtttggtatggcttcattcagctccggttcccaacgatcaaggcgagttacatgatcccccatgttgtgcaaaaaagcggttagctccttcggtcctccgatcgttgtcagaagtaagttggccgcagtgttatcactcatggttatggcagcactgcataattctcttactgtcatgccatccgtaagatgcttttctgtgactggtgagtactcaaccaagtcattctgagaatagtgtatgcggcgaccgagttgctcttgcccggcgtcaatacgggataataccgcgccacatagcagaactttaaaagtgctcatcattggaaaacgttcttcggggcgaaaactctcaaggatcttaccgctgttgagatccagttcgatgtaacccactcgtgcacccaactgatcttcagcatcttttactttcaccagcgtttctgggtgagcaaaaacaggaaggcaaaatgccgcaaaaaagggaataagggcgacacggaaatgttgaatactcatactcttcctttttcaatattattgaagcatttatcagggttattgtctcatgagcggatacatatttgaatgtatttagaaaaataaacaaataggggttccgcgcacatttccccgaaaagtgccacctgacgcgccctgtagcggcgcattaagcgcggcgggtgtggtggttacgcgcagcgtgaccgctacacttgccagcgccctagcgcccgctcctttcgctttcttcccttcctttctcgccacgttcgccggctttccccgtcaagctctaaatcgggggctccctttagggttccgatttagtgctttacggcacctcgaccccaaaaaacttgattagggtgatggttcacgtagtgggccatcgccctgatagacggtttttcgccctttgacgttggagtccacgttctttaatagtggactcttgttccaaactggaacaacactcaaccctatctcggtctattcttttgatttataagggattttgccgatttcggcctattggttaaaaaatgagctgatttaacaaaaatttaacgcgaattttaacaaaatattaacgcttacaattt

SEQ ID NO: 19 - DNA, 5893 bp, synthetic construct
  source 1..5893: mol_type = other DNA
ccattcgccattcaggctgcgcaactgttgggaagggcgatcggtgcgggcctcttcgctattacgccagctggcgaaagggggatgtgctgcaaggcgattaagttgggtaacgccagggttttcccagtcacgacgttgtaaaacgacggccagtgccaagctgatctatacattgaatcaatattggcaattagccatattagtcattggttatatagcataaatcaatattggctattggccattgcatacgttgtatctatatcataatatgtacatttatattggctcatgtccaatatgaccgccatgttgacattgattattgactagttattaatagtaatcaattacggggtcattagttcatagcccatatatggagttccgcgttacataacttacggtaaatggcccgcctggctgaccgcccaacgacccccgcccattgacgtcaataatgacgtatgttcccatagtaacgccaatagggactttccattgacgtcaatgggtggagtatttacggtaaactgcccacttggcagtacatcaagtgtatcatatgccaagtccgccccctattgacgtcaatgacggtaaatggcccgcctggcattatgcccagtacatgaccttacgggactttcctacttggcagtacatctacgtattagtcatcgctattaccatggtgatgcggttttggcagtacaccaatgggcgtggatagcggtttgactcacggggatttccaagtctccaccccattgacgtcaatgggagtttgttttggcaccaaaatcaacgggactttccaaaatgtcgtaataaccccgccccgttgacgcaaatgggcggtaggcgtgtacggtgggaggtctatataagcagagctcgtttagtgaaccgtcagaattaagcttgcggccgcgaattcatgtggcagttctctgctctactcctattcttcctcccaggctgctgcacggctcaggattcagtcacaggtccagaggaggtgagcggtcaggagcagggctccttgacagtgcagtgcagatattcctcatactggaagggttacaagaagtactggtgccgaggagttcctcagagatcatgtgatattcttgttgaaaccgataaatcagagcagctggtgaagaagaaccgtgtgtccatcagggacaaccagagagacttcatcttcacagtgaccatggaggatctgaggatgagcgatgctggcatttactggtgtggaattacgaaaggtggacctgatcccatgtttaaagttaatgtgaacattgaccaagccccaaaaagttcaatgatgaccaccacagccacagttctgaaatccatacaaccaagcgctgagaacactggcaaggaacaagtgactcagagcaaagaagtgactcagagcaggccccacaccaggtccctgctgagcagcatctacgtcgacatcgagggccgcatggaccccaaatcttgtaaaactcacacatgcccaccgtgcccagcacctgaactcctggggggaccgtcagtcttcctcttccccccaaaacccaaggacaccctcatgatctcccggacccctgaggtcacatgcgtggtggtggacgtgagccacgaagaccctgaggtcaagttcaactggtacgtggacggcgtggaggtgcataatgccaagacaaagccgcgggaggagcagtacaacagcacgtaccgtgtggtcagcgtcctcaccgtcctgcaccaggactggctgaatggcaaggagtacaagtgcaaggtctccaacaaagccctcccagcccccatcgagaaaaccatctccaaagccaaagggcagccccgagaaccacaggtgtacaccctgcccccatcccgggaggagatgaccaagaaccaggtcagcctgacctgcctggtcaaaggcttctatcccagcgacatcgccgtggagtgggagagcaatgggcagccggagaacaactacaagaccacgcctcccgtgctggactccgacggctccttcttcctctacagcaagctcaccgtggacaagagcaggtggcagcaggggaacgtcttctcatgctccgtgatgcacgaggctctgcacaaccactacacgcagaagagcctctccctgtctccgggtaaatgaggatcccgggctgattacaaggacgacgatgacaagtaggttgggtggcatccctgtgacccctccccagtgcctctcctggccctggaagttgccactccagtgcccaccagccttgtcctaataaaattaagttgcatcattttgtctgactaggtgtccttctataatattatggggtggaggggggtggtatggagcaaggggcaagttgggaagacaacctgtagggcctgcggggtctattgggaaccaagctggagtgcagtggcacaatcttggctcactgcaatctccgcctcctgggttcaagcgattctcctgcctcagcctcccgagttgttgggattccaggcatgcatgaccaggctcagctaatttttgtttttttggtagagacggggtttcaccatattggccaggctggtctccaactcctaatctcaggtgatctacccaccttggcctcccaaattgctgggattacaggcgtgaaccactgctcccttccctgtccttctgattttaaaataactataccagcaggaggacgtccagacacagcataggctacctggccatgcccaaccggtgggacatttgagttgcttgcttggcactgtcctctcatgcgttgggtccactcagtagatgcctgttgaattgggtacgcggccagcttggctgtggaatgtgtgtcagttagggtgtggaaagtccccaggctccccagcaggcagaagtatgcaaagcatgcatctcaattagtcagcaaccaggtgtggaaagtccccaggctccccagcaggcagaagtatgcaaagcatgcatctcaattagtcagcaaccatagtcccgcccctaactccgcccatcccgcccctaactccgcccagttccgcccattctccgccccatggctgactaattttttttatttatgcagaggccgaggccgcctcggcctctgagctattccagaagtagtgaggaggcttttttggaggcctaggcttttgcaaaaagctcctcgaggaactgaaaaaccagaaagttaattccctatagtgagtcgtattaaattcgtaatcatgtcatagctgtttcctgtgtgaaattgttatccgctcacaattccacacaacatacgagccggaagcataaagtgtaaagcctggggtgcctaatgagtgagctaactcacattaattgcgttgcgctcactgcccgctttccagtcgggaaacctgtcgtgccagctgcattaatgaatcggccaacgcgcggggagaggcggtttgcgtattgggcgctcttccgcttcctcgctcactgactcgctgcgctcggtcgttcggctgcggcgagcggtatcagctcactcaaaggcggtaatacggttatccacagaatcaggggataacgcaggaaagaacatgtgagcaaaaggccagcaaaaggccaggaaccgtaaaaaggccgcgttgctggcgtttttccataggctccgcccccctgacgagcatcacaaaaatcgacgctcaagtcagaggtggcgaaacccgacaggactataaagataccaggcgtttccccctggaagctccctcgtgcgctctcctgttccgaccctgccgcttaccggatacctgtccgcctttctcccttcgggaagcgtggcgctttctcatagctcacgctgtaggtatctcagttcggtgtaggtcgttcgctccaagctgggctgtgtgcacgaaccccccgttcagcccgaccgctgcgccttatccggtaactatcgtcttgagtccaacccggtaagacacgacttatcgccactggcagcagccactggtaacaggattagcagagcgaggtatgtaggcggtgctacagagttcttgaagtggtggcctaactacggctacactagaagaacagtatttggtatctgcgctctgctgaagccagttaccttcggaaaaagagttggtagctcttgatccggcaaacaaaccaccgctggtagcggtggtttttttgtttgcaagcagcagattacgcgcagaaaaaaaggatctcaagaagatcctttgatcttttctacggggtctgacgctcagtggaacgaaaactcacgttaagggattttggtcatgagattatcaaaaaggatcttcacctagatccttttaaattaaaaatgaagttttaaatcaatctaaagtatatatgagtaaacttggtctgacagttaccaatgcttaatcagtgaggcacctatctcagcgatctgtctatttcgttcatccatagttgcctgactccccgtcgtgtagataactacgatacgggagggcttaccatctggccccagtgctgcaatgataccgcgagacccacgctcaccggctccagatttatcagcaataaaccagccagccggaagggccgagcgcagaagtggtcctgcaactttatccgcctccatccagtctattaattgttgccgggaagctagagtaagtagttcgccagttaatagtttgcgcaacgttgttgccattgctacaggcatcgtggtgtcacgctcgtcgtttggtatggcttcattcagctccggttcccaacgatcaaggcgagttacatgatcccccatgttgtgcaaaaaagcggttagctccttcggtcctccgatcgttgtcagaagtaagttggccgcagtgttatcactcatggttatggcagcactgcataattctcttactgtcatgccatccgtaagatgcttttctgtgactggtgagtactcaaccaagtcattctgagaatagtgtatgcggcgaccgagttgctcttgcccggcgtcaatacgggataataccgcgccacatagcagaactttaaaagtgctcatcattggaaaacgttcttcggggcgaaaactctcaaggatcttaccgctgttgagatccagttcgatgtaacccactcgtgcacccaactgatcttcagcatcttttactttcaccagcgtttctgggtgagcaaaaacaggaaggcaaaatgccgcaaaaaagggaataagggcgacacggaaatgttgaatactcatactcttcctttttcaatattattgaagcatttatcagggttattgtctcatgagcggatacatatttgaatgtatttagaaaaataaacaaataggggttccgcgcacatttccccgaaaagtgccacctgacgcgccctgtagcggcgcattaagcgcggcgggtgtggtggttacgcgcagcgtgaccgctacacttgccagcgccctagcgcccgctcctttcgctttcttcccttcctttctcgccacgttcgccggctttccccgtcaagctctaaatcgggggctccctttagggttccgatttagtgctttacggcacctcgaccccaaaaaacttgattagggtgatggttcacgtagtgggccatcgccctgatagacggtttttcgccctttgacgttggagtccacgttctttaatagtggactcttgttccaaactggaacaacactcaaccctatctcggtctattcttttgatttataagggattttgccgatttcggcctattggttaaaaaatgagctgatttaacaaaaatttaacgcgaattttaacaaaatattaacgcttacaattt

SEQ ID NO: 20 - DNA, 20 bp, synthetic construct
  source 1..20: mol_type = other DNA
tcccaggttactccattgcc

SEQ ID NO: 21 - DNA, 20 bp, synthetic construct
  source 1..20: mol_type = other DNA
gcctgagccataagcacact

SEQ ID NO: 22 - DNA, 21 bp, synthetic construct
  source 1..21: mol_type = other DNA
tgtgggcatcaatggatttgg

SEQ ID NO: 23 - DNA, 22 bp, synthetic construct
  source 1..22: mol_type = other DNA
acaccatgtattccgggtcaat

SEQ ID NO: 24 - DNA, 24 bp, synthetic construct
  source 1..24: mol_type = other DNA
ttagaggaagttccctgttcaccc

SEQ ID NO: 25 - DNA, 24 bp, synthetic construct
  source 1..24: mol_type = other DNA
cttacctgggaggaagaataggag

SEQ ID NO: 26 - DNA, 23 bp, synthetic construct
  source 1..23: mol_type = other DNA
tgcagattcccacaatatgggag

SEQ ID NO: 27 - DNA, 23 bp, synthetic construct
  source 1..23: mol_type = other DNA
aacaggaagtgggtgctcttgag

SEQ ID NO: 28 - DNA, 38 bp, synthetic construct
  source 1..38: mol_type = other DNA
tgcggccgcgaattcgccaccatgtggctgtccccatc

SEQ ID NO: 29 - DNA, 37 bp, synthetic construct
  source 1..37: mol_type = other DNA
gtccccgctcaagagcacccacgtcgacatcgagggc

SEQ ID NO: 30 - DNA, 495 bp, synthetic construct
  source 1..495: mol_type = other DNA
atgtggctgtccccatctctgctgcttctcatcctcccaggttactccattgccgctaaaatcactggtccaacaacagtgaatggctcggagcagggctcattgactgtgcagtgtgcttatggctcaggctgggagacctacttgaagtggcggtgtcaaggagctgattggaattactgtaacatccttgttaaaacaaatggatcagagcaggaggtaaagaagaatcgagtttccatcagggacaatcagaaaaaccacgtgttcaccgtgaccatggagaatctcaaaagagatgatgctgacagttattggtgtgggactgagagacctggaattgatcttggggtcaaagttcaagtgaccattaacccaggcacacaaactgcagtctcagaatggacaaccacaacagcaagcctggctttcacagctgcagccacccagaagaccagcagccccctcaccaggtccccgctcaagagcacccac

SEQ ID NO: 31 - protein, 165 aa, synthetic construct
MWLSPSLLLLILPGYSIAAKITGPTTVNGSEQGSLTVQCAYGSGWETYLKWRCQGADWNYCNILVKTNGSEQEVKKNRVSIRDNQKNHVFTVTMENLKRDDADSYWCGTERPGIDLGVKVQVTINPGTQTAVSEWTTTTASLAFTAAATQKTSSPLTRSPLKSTH

SEQ ID NO: 32 - DNA, 5863 bp, synthetic construct
  source 1..5863: mol_type = other DNA
ccattcgccattcaggctgcgcaactgttgggaagggcgatcggtgcgggcctcttcgctattacgccagctggcgaaagggggatgtgctgcaaggcgattaagttgggtaacgccagggttttcccagtcacgacgttgtaaaacgacggccagtgccaagctgatctatacattgaatcaatattggcaattagccatattagtcattggttatatagcataaatcaatattggctattggccattgcatacgttgtatctatatcataatatgtacatttatattggctcatgtccaatatgaccgccatgttgacattgattattgactagttattaatagtaatcaattacggggtcattagttcatagcccatatatggagttccgcgttacataacttacggtaaatggcccgcctggctgaccgcccaacgacccccgcccattgacgtcaataatgacgtatgttcccatagtaacgccaatagggactttccattgacgtcaatgggtggagtatttacggtaaactgcccacttggcagtacatcaagtgtatcatatgccaagtccgccccctattgacgtcaatgacggtaaatggcccgcctggcattatgcccagtacatgaccttacgggactttcctacttggcagtacatctacgtattagtcatcgctattaccatggtgatgcggttttggcagtacaccaatgggcgtggatagcggtttgactcacggggatttccaagtctccaccccattgacgtcaatgggagtttgttttggcaccaaaatcaacgggactttccaaaatgtcgtaataaccccgccccgttgacgcaaatgggcggtaggcgtgtacggtgggaggtctatataagcagagctcgtttagtgaaccgtcagaattaagcttgcggccgcgaattcgccaccatgtggctgtccccatctctgctgcttctcatcctcccaggttactccattgccgctaaaatcactggtccaacaacagtgaatggctcggagcagggctcattgactgtgcagtgtgcttatggctcaggctgggagacctacttgaagtggcggtgtcaaggagctgattggaattactgtaacatccttgttaaaacaaatggatcagagcaggaggtaaagaagaatcgagtttccatcagggacaatcagaaaaaccacgtgttcaccgtgaccatggagaatctcaaaagagatgatgctgacagttattggtgtgggactgagagacctggaattgatcttggggtcaaagttcaagtgaccattaacccaggcacacaaactgcagtctcagaatggacaaccacaacagcaagcctggctttcacagctgcagccacccagaagaccagcagccccctcaccaggtccccgctcaagagcacccacgtcgacatcgagggccgcatggaccccaaatcttgtaaaactcacacatgcccaccgtgcccagcacctgaactcctggggggaccgtcagtcttcctcttccccccaaaacccaaggacaccctcatgatctcccggacccctgaggtcacatgcgtggtggtggacgtgagccacgaagaccctgaggtcaagttcaactggtacgtggacggcgtggaggtgcataatgccaagacaaagccgcgggaggagcagtacaacagcacgtaccgtgtggtcagcgtcctcaccgtcctgcaccaggactggctgaatggcaaggagtacaagtgcaaggtctccaacaaagccctcccagcccccatcgagaaaaccatctccaaagccaaagggcagccccgagaaccacaggtgtacaccctgcccccatcccgggaggagatgaccaagaaccaggtcagcctgacctgcctggtcaaaggcttctatcccagcgacatcgccgtggagtgggagagcaatgggcagccggagaacaactacaagaccacgcctcccgtgctggactccgacggctccttcttcctctacagcaagctcaccgtggacaagagcaggtggcagcaggggaacgtcttctcatgctccgtgatgcacgaggctctgcacaaccactacacgcagaagagcctctccctgtctccgggtaaatgaggatcccgggctgattacaaggacgacgatgacaagtaggttgggtggcatccctgtgacccctccccagtgcctctcctggccctggaagttgccactccagtgcccaccagccttgtcctaataaaattaagttgcatcattttgtctgactaggtgtccttctataatattatggggtggaggggggtggtatggagcaaggggcaagttgggaagacaacctgtagggcctgcggggtctattgggaaccaagctggagtgcagtggcacaatcttggctcactgcaatctccgcctcctgggttcaagcgattctcctgcctcagcctcccgagttgttgggattccaggcatgcatgaccaggctcagctaatttttgtttttttggtagagacggggtttcaccatattggccaggctggtctccaactcctaatctcaggtgatctacccaccttggcctcccaaattgctgggattacaggcgtgaaccactgctcccttccctgtccttctgattttaaaataactataccagcaggaggacgtccagacacagcataggctacctggccatgcccaaccggtgggacatttgagttgcttgcttggcactgtcctctcatgcgttgggtccactcagtagatgcctgttgaattgggtacgcggccagcttggctgtggaatgtgtgtcagttagggtgtggaaagtccccaggctccccagcaggcagaagtatgcaaagcatgcatctcaattagtcagcaaccaggtgtggaaagtccccaggctccccagcaggcagaagtatgcaaagcatgcatctcaattagtcagcaaccatagtcccgcccctaactccgcccatcccgcccctaactccgcccagttccgcccattctccgccccatggctgactaattttttttatttatgcagaggccgaggccgcctcggcctctgagctattccagaagtagtgaggaggcttttttggaggcctaggcttttgcaaaaagctcctcgaggaactgaaaaaccagaaagttaattccctatagtgagtcgtattaaattcgtaatcatgtcatagctgtttcctgtgtgaaattgttatccgctcacaattccacacaacatacgagccggaagcataaagtgtaaagcctggggtgcctaatgagtgagctaactcacattaattgcgttgcgctcactgcccgctttccagtcgggaaacctgtcgtgccagctgcattaatgaatcggccaacgcgcggggagaggcggtttgcgtattgggcgctcttccgcttcctcgctcactgactcgctgcgctcggtcgttcggctgcggcgagcggtatcagctcactcaaaggcggtaatacggttatccacagaatcaggggataacgcaggaaagaacatgtgagcaaaaggccagcaaaaggccaggaaccgtaaaaaggccgcgttgctggcgtttttccataggctccgcccccctgacgagcatcacaaaaatcgacgctcaagtcagaggtggcgaaacccgacaggactataaagataccaggcgtttccccctggaagctccctcgtgcgctctcctgttccgaccctgccgcttaccggatacctgtccgcctttctcccttcgggaagcgtggcgctttctcatagctcacgctgtaggtatctcagttcggtgtaggtcgttcgctccaagctgggctgtgtgcacgaaccccccgttcagcccgaccgctgcgccttatccggtaactatcgtcttgagtccaacccggtaagacacgacttatcgccactggcagcagccactggtaacaggattagcagagcgaggtatgtaggcggtgctacagagttcttgaagtggtggcctaactacggctacactagaagaacagtatttggtatctgcgctctgctgaagccagttaccttcggaaaaagagttggtagctcttgatccggcaaacaaaccaccgctggtagcggtggtttttttgtttgcaagcagcagattacgcgcagaaaaaaaggatctcaagaagatcctttgatcttttctacggggtctgacgctcagtggaacgaaaactcacgttaagggattttggtcatgagattatcaaaaaggatcttcacctagatccttttaaattaaaaatgaagttttaaatcaatctaaagtatatatgagtaaacttggtctgacagttaccaatgcttaatcagtgaggcacctatctcagcgatctgtctatttcgttcatccatagttgcctgactccccgtcgtgtagataactacgatacgggagggcttaccatctggccccagtgctgcaatgataccgcgagacccacgctcaccggctccagatttatcagcaataaaccagccagccggaagggccgagcgcagaagtggtcctgcaactttatccgcctccatccagtctattaattgttgccgggaagctagagtaagtagttcgccagttaatagtttgcgcaacgttgttgccattgctacaggcatcgtggtgtcacgctcgtcgtttggtatggcttcattcagctccggttcccaacgatcaaggcgagttacatgatcccccatgttgtgcaaaaaagcggttagctccttcggtcctccgatcgttgtcagaagtaagttggccgcagtgttatcactcatggttatggcagcactgcataattctcttactgtcatgccatccgtaagatgcttttctgtgactggtgagtactcaaccaagtcattctgagaatagtgtatgcggcgaccgagttgctcttgcccggcgtcaatacgggataataccgcgccacatagcagaactttaaaagtgctcatcattggaaaacgttcttcggggcgaaaactctcaaggatcttaccgctgttgagatccagttcgatgtaacccactcgtgcacccaactgatcttcagcatcttttactttcaccagcgtttctgggtgagcaaaaacaggaaggcaaaatgccgcaaaaaagggaataagggcgacacggaaatgttgaatactcatactcttcctttttcaatattattgaagcatttatcagggttattgtctcatgagcggatacatatttgaatgtatttagaaaaataaacaaataggggttccgcgcacatttccccgaaaagtgccacctgacgcgccctgtagcggcgcattaagcgcggcgggtgtggtggttacgcgcagcgtgaccgctacacttgccagcgccctagcgcccgctcctttcgctttcttcccttcctttctcgccacgttcgccggctttccccgtcaagctctaaatcgggggctccctttagggttccgatttagtgctttacggcacctcgaccccaaaaaacttgattagggtgatggttcacgtagtgggccatcgccctgatagacggtttttcgccctttgacgttggagtccacgttctttaatagtggactcttgttccaaactggaacaacactcaaccctatctcggtctattcttttgatttataagggattttgccgatttcggcctattggttaaaaaatgagctgatttaacaaaaatttaacgcgaattttaacaaaatattaacgcttacaattt

SEQ ID NO: 33 - protein, 415 aa, synthetic construct
MWQFSALLLFFLPGCCTAQDSVTGPEEVSGQEQGSLTVQCRYSSYWKGYKKYWCRGVPQRSCDILVETDKSEQLVKKNRVSIRDNQRDFIFTVTMEDLRMSDAGIYWCGITKGGPDPMFKVNVNIDQAPKSSMMTTTATVLKSIQPSAENTGKEQVTQSKEVTQSRPHTRSLLSSIYVDIEGRMDPKSCKTHTCPPCPAPELLGGPSVFLFPPKPKDTLMISRTPEVTCVVVDVSHEDPEVKFNWYVDGVEVHNAKTKPREEQYNSTYRVVSVLTVLHQDWLNGKEYKCKVSNKALPAPIEKTISKAKGQPREPQVYTLPPSREEMTKNQVSLTCLVKGFYPSDIAVEWESNGQPENNYKTTPPVLDSDGSFFLYSKLTVDKSRWQQGNVFSCSVMHEALHNHYTQKSLSLSPGK

SEQ ID NO: 34 - protein, 403 aa, synthetic construct
MWLSPSLLLLILPGYSIAAKITGPTTVNGSEQGSLTVQCAYGSGWETYLKWRCQGADWNYCNILVKTNGSEQEVKKNRVSIRDNQKNHVFTVTMENLKRDDADSYWCGTERPGIDLGVKVQVTINPGTQTAVSEWTTTTASLAFTAAATQKTSSPLTRSPLKSTHVDIEGRMDPKSCKTHTCPPCPAPELLGGPSVFLFPPKPKDTLMISRTPEVTCVVVDVSHEDPEVKFNWYVDGVEVHNAKTKPREEQYNSTYRVVSVLTVLHQDWLNGKEYKCKVSNKALPAPIEKTISKAKGQPREPQVYTLPPSREEMTKNQVSLTCLVKGFYPSDIAVEWESNGQPENNYKTTPPVLDSDGSFFLYSKLTVDKSRWQQGNVFSCSVMHEALHNHYTQKSLSLSPGK